European Patent Application EP 4 410 984 A1, published August 7, 2024. Title: GENETICALLY ENGINEERED STRAIN FOR PRODUCING POLYLACTIC ACID AND METHOD FOR PRODUCING POLYLACTIC ACID. Applicant: SHANGHAI SIPENG TECHNOLOGY LTD. The sequence listing filed with the application follows.

SEQUENCE LISTING (21 sequences)

SEQ ID NO: 1 - DNA, 31 bp, synthetic construct
  source 1..31: mol_type = other DNA
actcgagatgagcaacaagtcaaatgatgaa

SEQ ID NO: 2 - DNA, 31 bp, synthetic construct
  source 1..31: mol_type = other DNA
ggatcctctaggacttcatttctttcaggcc

SEQ ID NO: 3 - DNA, 19 bp, synthetic construct
  source 1..19: mol_type = other DNA
acctggaattggttgaagg

SEQ ID NO: 4 - DNA, 18 bp, synthetic construct
  source 1..18: mol_type = other DNA
acagccaagcttgcatgc

SEQ ID NO: 5 - DNA, 18 bp, synthetic construct
  source 1..18: mol_type = other DNA
cgactgcacggtgcacca

SEQ ID NO: 6 - DNA, 22 bp, synthetic construct
  source 1..22: mol_type = other DNA
catggtctgtttcctgtgtgaa

SEQ ID NO: 7 - DNA, 24 bp, synthetic construct
  source 1..24: mol_type = other DNA
tatcaataagtattaggtatatgg

SEQ ID NO: 8 - DNA, 22 bp, synthetic construct
  source 1..22: mol_type = other DNA
atgtatttgtcgatgttcagat

SEQ ID NO: 9 - DNA, 20 bp, synthetic construct
  source 1..20: mol_type = other DNA
acctgtagagaagagtccct

SEQ ID NO: 10 - DNA, 25 bp, synthetic construct
  source 1..25: mol_type = other DNA
tgaattaatctcctacttgacttta

SEQ ID NO: 11 - DNA, 26 bp, synthetic construct
  source 1..26: mol_type = other DNA
actagtatggctgcacctgtcacgaa

SEQ ID NO: 12 - DNA, 30 bp, synthetic construct
  source 1..30: mol_type = other DNA
ggatccttagtcactgctttccagaaacac

SEQ ID NO: 13 - DNA, 18 bp, synthetic construct
  source 1..18: mol_type = other DNA
agggcttcccggtatcaa

SEQ ID NO: 14 - DNA, 18 bp, synthetic construct
  source 1..18: mol_type = other DNA
acagccaagcttgcatgc

SEQ ID NO: 15 - DNA, 30 bp, synthetic construct
  source 1..30: mol_type = other DNA
ggatcctatcaataagtattaggtatatgg

SEQ ID NO: 16 - DNA, 24 bp, synthetic construct
  source 1..24: mol_type = other DNA
gaattcgctgtcgaagttgaacat

SEQ ID NO: 17 - DNA, 30 bp, synthetic construct
  source 1..30: mol_type = other DNA
gaattctatcaataagtattaggtatatgg

SEQ ID NO: 18 - DNA, 24 bp, synthetic construct
  source 1..24: mol_type = other DNA
gagctcgctgtcgaagttgaacat

SEQ ID NO: 19 - DNA, 16 bp, synthetic construct
  source 1..16: mol_type = other DNA
aagaaggagatatacc

SEQ ID NO: 20 - DNA, 686 bp, synthetic construct
  source 1..686: mol_type = other DNA
tatcaataagtattaggtatatggatcataattgtatgcccgactattgcttaaactgactgaccactgaccttaagagtaatggcgtgcaaggcccagtgatcaatttcattatttttcattatttcatctccattgtccctgaaaatcagttgtgtcgcccctctacacagcccagaactatggtaaaggcgcacgaaaaaccgccaggtaaactcttctcaacccccaaaacgccctctgtttacccatggaaaaaacgacaattacaagaaagtaaaacttatgtcatctataagcttcgtgtatattaacttcctgttacaaagctttacaaaactctcattaatcctttagactaagtttagtcagttccaatctgaacatcgacaaatacatcctgcgatcgctgctatccagcattttctgttgggccattgcattgccactgattttccaacatataaaaagacaagcccgaacagtcgtccgggctttttttggtaccccggtgtttggattgtcggagttgtactcgtccgttaaggatgaacagttcttcggggttgagtctgctaactaattagccattaacagcggcttaactaacagttagtcattggcaattgtcaaaaaattgttaatcagccaaaacccactgcttactgatgttcaacttcgacagc

SEQ ID NO: 21 - DNA, 2084 bp, synthetic construct
  source 1..2084: mol_type = other DNA
tatcaataagtattaggtatatggatcataattgtatgcccgactattgcttaaactgactgaccactgaccttaagagtaatggcgtgcaaggcccagtgatcaatttcattatttttcattatttcatctccattgtccctgaaaatcagttgtgtcgcccctctacacagcccagaactatggtaaaggcgcacgaaaaaccgccaggtaaactcttctcaacccccaaaacgccctctgtttacccatggaaaaaacgacaattacaagaaagtaaaacttatgtcatctataagcttcgtgtatattaacttcctgttacaaagctttacaaaactctcattaatcctttagactaagtttagtcagttccaatctgaacatcgacaaatacatgatcaggatcttgttgaaacgcattttctgttgggccattgcattgccactgattttccaacatataaaaagacaagcccgaacagtcgtccgggctttttttggtaccccggtgtttggattgtcggagttgtactcgtccgttaaggatgaacagttcttcggggttgagtctgctaactaattagccattaacagcggcttaactaacagttagtcattggcaattgtcaaaaaattgttaatcagccaaaacccactgcttactgatgttcaacttcgacagcgagctggaattctatcaataagtattaggtatatggatcataattgtatgcccgactattgcttaaactgactgaccactgaccttaagagtaatggcgtgcaaggcccagtgatcaatttcattatttttcattatttcatctccattgtccctgaaaatcagttgtgtcgcccctctacacagcccagaactatggtaaaggcgcacgaaaaaccgccaggtaaactcttctcaacccccaaaacgccctctgtttacccatggaaaaaacgacaattacaagaaagtaaaacttatgtcatctataagcttcgtgtatattaacttcctgttacaaagctttacaaaactctcattaatcctttagactaagtttagtcagttccaatctgaacatcgacaaatacatacgctggcgtccggtttcagtcattttctgttgggccattgcattgccactgattttccaacatataaaaagacaagcccgaacagtcgtccgggctttttttggtaccccggtgtttggattgtcggagttgtactcgtccgttaaggatgaacagttcttcggggttgagtctgctaactaattagccattaacagcggcttaactaacagttagtcattggcaattgtcaaaaaattgttaatcagccaaaacccactgcttactgatgttcaacttcgacagcgcggccgctatcaataagtattaggtatatggatcataattgtatgcccgactattgcttaaactgactgaccactgaccttaagagtaatggcgtgcaaggcccagtgatcaatttcattatttttcattatttcatctccattgtccctgaaaatcagttgtgtcgcccctctacacagcccagaactatggtaaaggcgcacgaaaaaccgccaggtaaactcttctcaacccccaaaacgccctctgtttacccatggaaaaaacgacaattacaagaaagtaaaacttatgtcatctataagcttcgtgtatattaacttcctgttacaaagctttacaaaactctcattaatcctttagactaagtttagtcagttccaatctgaacatcgacaaatacatgttgaggctgccatcactgcgcattttctgttgggccattgcattgccactgattttccaacatataaaaagacaagcccgaacagtcgtccgggctttttttggtaccccggtgtttggattgtcggagttgtactcgtccgttaaggatgaacagttcttcggggttgagtctgctaactaattagccattaacagcggcttaactaacagttagtcattggcaattgtcaaaaaattgttaatcagccaaaacccactgcttactgatgttcaacttcgacagcggatcc